European Patent Application EP 4 623 911 A1, published October 1, 2025. Title: PI4KB inhibitors for the treatment of fatty liver disease. Applicant: ETH Zürich. Application EP. The sequence listing filed with the application follows.

SEQUENCE LISTING (82 sequences)

SEQ ID NO: 1 - RNA, 19 nt, synthetic construct
  source 1..19: mol_type = other RNA; note = siRNA targeting murine gene Pi4kb
ccaagttacggaagctaat

SEQ ID NO: 2 - RNA, 19 nt, synthetic construct
  source 1..19: mol_type = other RNA; note = siRNA targeting murine gene Pi4kb
gcccaattatgacaatgat

SEQ ID NO: 3 - RNA, 19 nt, synthetic construct
  source 1..19: mol_type = other RNA; note = siRNA for murine gene Sacm1l
gcatctgaagctgcatatt

SEQ ID NO: 4 - RNA, 19 nt, synthetic construct
  source 1..19: mol_type = other RNA; note = siRNA targeting murine gene Sacm1l
ggtggcaggtaattatctt

SEQ ID NO: 5 - RNA, 19 nt, synthetic construct
  source 1..19: mol_type = other RNA; note = siRNA targeting murine gene Cul7
ggaagaagccattggagaa

SEQ ID NO: 6 - RNA, 19 nt, synthetic construct
  source 1..19: mol_type = other RNA; note = siRNA targeting murine gene Fbxw8
gatccatgcctatgaattt

SEQ ID NO: 7 - RNA, 19 nt, synthetic construct
  source 1..19: mol_type = other RNA; note = siRNA targeting Human gene PI4KB
gggatgaccttcggcaaga

SEQ ID NO: 8 - RNA, 19 nt, synthetic construct
  source 1..19: mol_type = other RNA; note = siRNA targeting Human gene SACM1L
gcctattatcatggttgtt

SEQ ID NO: 9 - RNA, 19 nt, synthetic construct
  source 1..19: mol_type = other RNA; note = siRNA targeting Human gene CUL7
gcacaagagcgagaaggaa

SEQ ID NO: 10 - RNA, 19 nt, synthetic construct
  source 1..19: mol_type = other RNA; note = siRNA targeting Human gene CUL7
tgagatcctagctgaactg

SEQ ID NO: 11 - RNA, 19 nt, synthetic construct
  source 1..19: mol_type = other RNA; note = siRNA targeting Human gene FBXW8
gggattatcggatgaacca

SEQ ID NO: 12 - RNA, 19 nt, synthetic construct
  source 1..19: mol_type = other RNA; note = siRNA targeting Human gene FBXW8
gggatttaaggaccggaaa

SEQ ID NO: 13 - RNA, 19 nt, synthetic construct
  source 1..19: mol_type = other RNA; note = siRNA targeting Human gene HACE1
tatagcgctgatgtcaaca

SEQ ID NO: 14 - RNA, 19 nt, synthetic construct
  source 1..19: mol_type = other RNA; note = siRNA targeting Human gene STUB1
cgctggtggccgtgtatta

SEQ ID NO: 15 - RNA, 19 nt, synthetic construct
  source 1..19: mol_type = other RNA; note = siRNA targeting Human gene SH3RF1
cagaggccttggaaacctg

SEQ ID NO: 16 - RNA, 19 nt, synthetic construct
  source 1..19: mol_type = other RNA; note = siRNA targeting Human gene KLHL20
gcctgctgtgaattcttaa

SEQ ID NO: 17 - RNA, 19 nt, synthetic construct
  source 1..19: mol_type = other RNA; note = siRNA targeting Human gene PJA2
gagatgagtttgaagagtt

SEQ ID NO: 18 - RNA, 19 nt, synthetic construct
  source 1..19: mol_type = other RNA; note = siRNA targeting Human gene CUL3
gagaagatgtactaaattc

SEQ ID NO: 19 - RNA, 19 nt, synthetic construct
  source 1..19: mol_type = other RNA; note = siRNA targeting Human gene CUL5
gacacgacgtcttatatta

SEQ ID NO: 20 - RNA, 19 nt, synthetic construct
  source 1..19: mol_type = other RNA; note = siRNA targeting Human gene ASB13
ggagaagattgccaagtta

SEQ ID NO: 21 - RNA, 19 nt, synthetic construct
  source 1..19: mol_type = other RNA; note = siRNA targeting Human gene FBXL14
gctacaacctcaccgacaa

SEQ ID NO: 22 - RNA, 19 nt, synthetic construct
  source 1..19: mol_type = other RNA; note = siRNA targeting Human gene FBXW4
ggatgcagctagaggatga

SEQ ID NO: 23 - RNA, 19 nt, synthetic construct
  source 1..19: mol_type = other RNA; note = siRNA targeting Human gene HERC1
cggcatggatgaacaaatt

SEQ ID NO: 24 - RNA, 19 nt, synthetic construct
  source 1..19: mol_type = other RNA; note = siRNA targeting Human gene KBTBD8
gagcatgaacagaatgaaa

SEQ ID NO: 25 - RNA, 19 nt, synthetic construct
  source 1..19: mol_type = other RNA; note = siRNA targeting Human gene UBAC
agagatgagctgacggaaa

SEQ ID NO: 26 - RNA, 19 nt, synthetic construct
  source 1..19: mol_type = other RNA; note = siRNA targeting Human gene RNF121
ccttctcatctctggccga

SEQ ID NO: 27 - RNA, 19 nt, synthetic construct
  source 1..19: mol_type = other RNA; note = siRNA targeting Human gene HECW1
cagctgcaattccgatttg

SEQ ID NO: 28 - RNA, 19 nt, synthetic construct
  source 1..19: mol_type = other RNA; note = siRNA targeting Human gene HECW2
gtgggtacctccagtttaa

SEQ ID NO: 29 - RNA, 19 nt, synthetic construct
  source 1..19: mol_type = other RNA; note = siRNA targeting Human gene NEDD4
ggcgatttgtaaaccgaat

SEQ ID NO: 30 - RNA, 19 nt, synthetic construct
  source 1..19: mol_type = other RNA; note = siRNA targeting Human gene NEDD4L
gaatatcgctggagactct

SEQ ID NO: 31 - RNA, 19 nt, synthetic construct
  source 1..19: mol_type = other RNA; note = siRNA targeting Human gene NEDD4L
gagtcctatcggagaatta

SEQ ID NO: 32 - RNA, 19 nt, synthetic construct
  source 1..19: mol_type = other RNA; note = siRNA targeting Human gene SMURF1
gggctcttccagtattcta

SEQ ID NO: 33 - RNA, 19 nt, synthetic construct
  source 1..19: mol_type = other RNA; note = siRNA targeting Human gene SMURF2
gatgagaacactccaatta

SEQ ID NO: 34 - RNA, 19 nt, synthetic construct
  source 1..19: mol_type = other RNA; note = siRNA targeting Human gene ITCH
gctgttgtttgccatagaa

SEQ ID NO: 35 - RNA, 19 nt, synthetic construct
  source 1..19: mol_type = other RNA; note = siRNA targeting Human gene COP1
gctgtggtctaccaatcta

SEQ ID NO: 36 - RNA, 19 nt, synthetic construct
  source 1..19: mol_type = other RNA; note = siRNA targeting Human gene CBLC
gggaaagtactgtggacac

SEQ ID NO: 37 - RNA, 19 nt, synthetic construct
  source 1..19: mol_type = other RNA; note = siRNA targeting Human gene HECTD3
gcgggaactagggttgaat

SEQ ID NO: 38 - RNA, 19 nt, synthetic construct
  source 1..19: mol_type = other RNA; note = siRNA targeting Human gene OSBP1
cacaactgtacacaacatt

SEQ ID NO: 39 - RNA, 19 nt, synthetic construct
  source 1..19: mol_type = other RNA; note = siRNA targeting Human gene CRET
gaagatgactttcctacaa

SEQ ID NO: 40 - RNA, 19 nt, synthetic construct
  source 1..19: mol_type = other RNA; note = siRNA targeting Human gene ORP1
gccagtgccggattctgaa

SEQ ID NO: 41 - RNA, 19 nt, synthetic construct
  source 1..19: mol_type = other RNA; note = siRNA targeting Human gene ORP5
tgggtgggaaggtcaccat

SEQ ID NO: 42 - RNA, 19 nt, synthetic construct
  source 1..19: mol_type = other RNA; note = siRNA targeting Human gene ORP9
gaggagcacaagagcgtta

SEQ ID NO: 43 - RNA, 19 nt, synthetic construct
  source 1..19: mol_type = other RNA; note = siRNA targeting Human gene ORP10
caacccaaccaacaccatt

SEQ ID NO: 44 - RNA, 19 nt, synthetic construct
  source 1..19: mol_type = other RNA; note = siRNA targeting Human gene ORP11
gagacttaattagacgaat

SEQ ID NO: 45 - RNA, 19 nt, synthetic construct
  source 1..19: mol_type = other RNA; note = siRNA targeting Human gene VAPA
ggcaaaacctgatgaatta

SEQ ID NO: 46 - RNA, 19 nt, synthetic construct
  source 1..19: mol_type = other RNA; note = siRNA targeting Human gene VAPB
gtaagaggctgcaaggtga

SEQ ID NO: 47 - RNA, 19 nt, synthetic construct
  source 1..19: mol_type = other RNA; note = siRNA targeting Human gene FAPP1
cgaagaacctactcagata

SEQ ID NO: 48 - RNA, 19 nt, synthetic construct
  source 1..19: mol_type = other RNA; note = siRNA targeting Human gene FAPP2
gagatagactgcagcatat

SEQ ID NO: 49 - RNA, 19 nt, synthetic construct
  source 1..19: mol_type = other RNA; note = siRNA targeting Human gene GOLPH3
gttaagaaatgtacgggaa

SEQ ID NO: 50 - RNA, 19 nt, synthetic construct
  source 1..19: mol_type = other RNA; note = siRNA targeting Human gene GP73
gcatcatcgtcttgggctt

SEQ ID NO: 51 - RNA, 19 nt, synthetic construct
  source 1..19: mol_type = other RNA; note = siRNA targeting Human gene GP73
gcaggatgtcctccagttt

SEQ ID NO: 52 - RNA, 19 nt, synthetic construct
  source 1..19: mol_type = other RNA; note = siRNA targeting Human gene GP73
gccagtgcatcaatcagat

SEQ ID NO: 53 - RNA, 19 nt, synthetic construct
  source 1..19: mol_type = other RNA; note = siRNA targeting Human gene GP73
ggattcaaagagacaagtt

SEQ ID NO: 54 - RNA, 19 nt, synthetic construct
  source 1..19: mol_type = other RNA; note = siRNA targeting Human gene ATGL
gcgagaagacgtggaacat

SEQ ID NO: 55 - RNA, 19 nt, synthetic construct
  source 1..19: mol_type = other RNA; note = siRNA targeting Human gene ATGL
cctgccactctatgagctt

SEQ ID NO: 56 - RNA, 19 nt, synthetic construct
  source 1..19: mol_type = other RNA; note = siRNA targeting Human gene ATGL
gcacctgtgccttaatctt

SEQ ID NO: 57 - DNA, 24 bp, synthetic construct
  source 1..24: mol_type = other DNA; note = primer targeting murine gene Emr1
cagctgtaaccggatggcaaactt

SEQ ID NO: 58 - DNA, 23 bp, synthetic construct
  source 1..23: mol_type = other DNA; note = primer targeting murine gene Emr1
tgaacagcacgacacagcaggaa

SEQ ID NO: 59 - DNA, 18 bp, synthetic construct
  source 1..18: mol_type = other DNA; note = primer targeting murine gene Ccl2
catccacgtgttggctca

SEQ ID NO: 60 - DNA, 23 bp, synthetic construct
  source 1..23: mol_type = other DNA; note = primer targeting murine gene Ccl2
gatcatcttgctggtgaatgagt

SEQ ID NO: 61 - DNA, 20 bp, synthetic construct
  source 1..20: mol_type = other DNA; note = primer targeting murine gene Tnf-alpha
caggggccaccacgctcttc

SEQ ID NO: 62 - DNA, 24 bp, synthetic construct
  source 1..24: mol_type = other DNA; note = primer targeting murine gene Tnf-alpha
tacgacgtgggctacaggcttgtc

SEQ ID NO: 63 - DNA, 19 bp, synthetic construct
  source 1..19: mol_type = other DNA; note = primer targeting murine gene Il1b
agttgacggaccccaaaag

SEQ ID NO: 64 - DNA, 20 bp, synthetic construct
  source 1..20: mol_type = other DNA; note = primer targeting murine gene Il1b
agctggatgctctcatcagg

SEQ ID NO: 65 - DNA, 20 bp, synthetic construct
  source 1..20: mol_type = other DNA; note = primer targeting murine gene Tgfb1
gctgaaccaaggagacggaa

SEQ ID NO: 66 - DNA, 20 bp, synthetic construct
  source 1..20: mol_type = other DNA; note = primer targeting murine gene Tgfb1
atgtcatggatggtgcccag

SEQ ID NO: 67 - DNA, 21 bp, synthetic construct
  source 1..21: mol_type = other DNA; note = primer targeting murine gene Col1a1
catgttcagctttgtggacct

SEQ ID NO: 68 - DNA, 20 bp, synthetic construct
  source 1..20: mol_type = other DNA; note = primer targeting murine gene Col1a1
gcagctgacttcagggatgt

SEQ ID NO: 69 - DNA, 22 bp, synthetic construct
  source 1..22: mol_type = other DNA; note = primer targeting murine gene Col1a2
gcaggttcacctactctgtcct

SEQ ID NO: 70 - DNA, 20 bp, synthetic construct
  source 1..20: mol_type = other DNA; note = primer targeting murine gene Col1a2
cttgccccattcatttgtct

SEQ ID NO: 71 - DNA, 24 bp, synthetic construct
  source 1..24: mol_type = other DNA; note = primer targeting murine gene Timp1
gatatgcccacaagtcccagaacc

SEQ ID NO: 72 - DNA, 23 bp, synthetic construct
  source 1..23: mol_type = other DNA; note = primer targeting murine gene Timp1
gcacaccccacagccagcactat

SEQ ID NO: 73 - DNA, 20 bp, synthetic construct
  source 1..20: mol_type = other DNA; note = primer targeting murine gene Acta2
actgggacgacatggaaaag

SEQ ID NO: 74 - DNA, 20 bp, synthetic construct
  source 1..20: mol_type = other DNA; note = primer targeting murine gene Acta2
gttcagtggtgcctctgtca

SEQ ID NO: 75 - DNA, 19 bp, synthetic construct
  source 1..19: mol_type = other DNA; note = primer targeting murine gene Atgl
tgaccatctgccttccaga

SEQ ID NO: 76 - DNA, 18 bp, synthetic construct
  source 1..18: mol_type = other DNA; note = primer targeting murine gene Atgl
tgtaggtggcgcaagaca

SEQ ID NO: 77 - DNA, 20 bp, synthetic construct
  source 1..20: mol_type = other DNA; note = primer targeting murine gene 36B4
gccgtgatgcccagggaaga

SEQ ID NO: 78 - DNA, 21 bp, synthetic construct
  source 1..21: mol_type = other DNA; note = primer targeting murine gene 36B4
catctgcttggagcccacgtt

SEQ ID NO: 79 - DNA, 19 bp, synthetic construct
  source 1..19: mol_type = other DNA; note = primer targeting Human gene ATGL
ctccaccaacatccacgag

SEQ ID NO: 80 - DNA, 19 bp, synthetic construct
  source 1..19: mol_type = other DNA; note = primer targeting Human gene ATGL
ccctgcttgcacatctctc

SEQ ID NO: 81 - DNA, 20 bp, synthetic construct
  source 1..20: mol_type = other DNA; note = primer targeting Human gene 36B4
ccaggcgtcctcgtggaagt

SEQ ID NO: 82 - DNA, 22 bp, synthetic construct
  source 1..22: mol_type = other DNA; note = primer targeting Human gene 36B4
tgctgcatctgcttggagccca